European Patent Specification EP 3 966 226 B1, published December 24, 2025. Title: MASP inhibitory compounds and uses thereof. Applicant: Bayer AG Bayer Pharma AG. The sequence listing filed with the application follows.

SEQUENCE LISTING (10 sequences)

SEQ ID NO: 1 - protein, 14 aa, Artificial Sequence
  SFMI-1
  DISULFID (3)..(11): disulfide bond;
  DISULFID (3)..(11): disulfide bond
GICSRSLPPICIPD

SEQ ID NO: 2 - protein, 430 aa, Artificial Sequence
  MASP-1_Human_Sequence fragment_C-terminal His Tag and N-terminal Ig-kappa secretion signal
METDTLLLWVLLLWVPGSTGDAGNECPELQPPVHGKIEPSQAKYFFKDQVLVSCDTGYKVLKDNVEMDTFQIECLKDGTWSNKIPTCKIVDCRAPGELEHGLITFSTRNNLTTYKSEIKYSCQEPYYKMLNNNTGIYTCSAQGVWMNKVLGRSLPTCLPVCGLPKFSRKLMARIFNGRPAQKGTTPWIAMLSHLNGQPFCGGSLLGSSWIVTAAHCLHQSLDPEDPTLRDSDLLSPSDFKIILGKHWRLRSDENEQHLGVKHTTLHPQYDPNTFENDVALVELLESPVLNAFVMPICLPEGPQQEGAMVIVSGWGKQFLQRFPETLMEIEIPIVDHSTCQKAYAPLKKKVTRDMICAGEKEGGKDACAGDSGGPMVTLNRERGQWYLVGTVSWGDDCGKKDRYGVYSYIHHNKDWIQRVTGVRNHHHHHH

SEQ ID NO: 3 - protein, 417 aa, Artificial Sequence
  MASP-2_Human_Sequence fragment_C-terminal His Tag and N-terminal Ig-kappa secretion signal
METDTLLLWVLLLWVPGSTGDAQPCPYPMAPPNGHVSPVQAKYILKDSFSIFCETGYELLQGHLPLKSFTAVCQKDGSWDRPMPACSIVDCGPPDDLPSGRVEYITGPGVTTYKAVIQYSCEETFYTMKVNDGKYVCEADGFWTSSKGEKSLPVCEPVCGLSARTTGGRIYGGQKAKPGDFPWQVLILGGTTAAGALLYDNWVLTAAHAVYEQKHDASALDIRMGTLKRLSPHYTQAWSEAVFIHEGYTHDAGFDNDIALIKLNNKVVINSNITPICLPRKEAESFMRTDDIGTASGWGLTQRGFLARNLMYVDIPIVDHQKCTAAYEKPPYPRGSVTANMLCAGLESGGKDSCRGDSGGALVFLDSETERWFVGGIVSWGSMNCGEAGQYGVYTKVINYIPWIENIISDFHHHHHH

SEQ ID NO: 4 - protein, 430 aa, Artificial Sequence
  MASP-1_Rat_Sequence fragment_C-terminal His Tag and N-terminal Ig-kappa secretion signal
METDTLLLWVLLLWVPGSTGDAGNECPKLQPPVYGKIEPSQAVYSFKDQVLISCDTGYKVLKDNEVMDTFQIECLKDGAWSNKIPTCKIVDCGVPAVLKHGLVTFSTRNNLTTYKSEIRYSCQQPYYKMLHNTTGVYTCSAHGTWTNEVLKRSLPTCLPVCGLPKFSRKHISRIFNGRPAQKGTTPWIAMLSQLNGQPFCGGSLLGSNWVLTAAHCLHHPLDPEEPILHNSHLLSPSDFKIIMGKHWRRRSDEDEQHLHVKHIMLHPLYNPSTFENDLGLVELSESPRLNDFVMPVCLPEHPSTEGTMVIVSGWGKQFLQRLPENLMEIEIPIVNYHTCQEAYTPLGKKVTQDMICAGEKEGGKDACAGDSGGPMVTKDAERDQWYLVGVVSWGEDCGKKDRYGVYSYIYPNKDWIQRVTGVRNHHHHHH

SEQ ID NO: 5 - protein, 417 aa, Artificial Sequence
  MASP-2_Rat_Sequence fragment_C-terminal His Tag and N-terminal Ig-kappa secretion signal
METDTLLLWVLLLWVPGSTGDTAQPCPDPTAPPNGHISPVQATYVLKDSFSVFCKTGFELLQGSVPLKSFTAVCQKDGSWDRPIPECSIIDCGPPDDLPNGHVDYITGPEVTTYKAVIQYSCEETFYTMSSNGKYVCEADGFWTSSKGEKSLPVCKPVCGLSTHTSGGRIIGGQPAKPGDFPWQVLLLGETTAAGALIHDDWVLTAAHAVYGKTEAMSSLDIRMGILKRLSLIYTQAWPEAVFIHEGYTHGAGFDNDIALIKLKNKVTINRNIMPICLPRKEAASLMKTDFVGTVAGWGLTQKGFLARNLMFVDIPIVDHQKCATAYTKQPYPGAKVTVNMLCAGLDRGGKDSCRGDSGGALVFLDNETQRWFVGGIVSWGSINCGGSEQYGVYTKVTNYIPWIENIINNFHHHHHH

SEQ ID NO: 6 - protein, 11 aa, Artificial Sequence
  Fluorescence Resonance Energy Transfer substrate
  Xaa (1)..(1): Xaa is 2-aminobenzoyl
  MOD_RES (10)..(10): AMIDATION
  Xaa (11)..(11): Xaa is a non peptidic capping group (2,4-dinitrophenyl; bound to lysine amino group on position 6)
XMYGGARRLKX

SEQ ID NO: 7 - protein, 13 aa, Artificial Sequence
  Fluorescence resonance energy transfer substrate
  Xaa (1)..(1): Xaa is 4-((4-(dimethylamino)phenyl)azo)benzoic acid
  MOD_RES (12)..(12): AMIDATION
  Xaa (13)..(13): Xaa is 5-[(2-Aminoethyl) amino]naphthalene-1-sulfonyl (bound to Glutamic acid caboxylic acid group on position 5)
XKISPQGYGRREX

SEQ ID NO: 8 - protein, 11 aa, Artificial Sequence
  Fluorescence resonance energy transfer substrate
  Xaa (1)..(1): Xaa is 4-((4-(dimethylamino)phenyl)azo)benzoic acid
  MOD_RES (10)..(10): AMIDATION
  Xaa (11)..(11): Xaa is 5-[(2-Aminoethyl) amino]naphthalene-1-sulfonyl (bound to Glutamic acid caboxylic acid group on position 5)
XMYGGARRLEX

SEQ ID NO: 9 - protein, 11 aa, Artificial Sequence
  Fluorescence resonance energy transfer substrate
  Xaa (1)..(1): Xaa is 2-aminobenzoyl
  MOD_RES (10)..(10): AMIDATION
  Xaa (11)..(11): Xaa is a non peptidic capping group (2,4-dinitrophenyl; bound to lysine amino group on position 6)
XIEGRTSEDKX

SEQ ID NO: 10 - protein, 14 aa, Artificial Sequence
  Ala-1 SFMI-1
  DISULFID (3)..(11)
  DISULFID (3)..(11): disulfide bond
AICSRSLPPICIPD